European Patent Application EP 4 563 148 A1, published June 4, 2025. Title: がんを治療するための医薬. Applicant: 株式会社サイエンステクノロジーインタラクト. The sequence listing filed with the application follows.

SEQUENCE LISTING (3 sequences)

SEQ ID NO: 1 - DNA, 22 bp, synthetic construct
  source 1..22: mol_type = other DNA
gtcctgctggagttcgtgaccg

SEQ ID NO: 2 - DNA, 20 bp, synthetic construct
  source 1..20: mol_type = other DNA
gtgcaatcaaagtcctcggc

SEQ ID NO: 3 - DNA, 22 bp, synthetic construct
  source 1..22: mol_type = other DNA
agttgcgttacaccctttcttg